European Patent Specification EP 3 397 969 B1, published September 6, 2023. Title: METHODS FOR MASS SPECTROMETRY-BASED STRUCTURE DETERMINATION OF BIOMACROMOLECULES. Applicant: VITO NV & UNIVERSITEIT ANTWERPEN. The sequence listing filed with the application follows.

SEQUENCE LISTING (4 sequences)

SEQ ID NO: 1 - protein, 151 aa, Homo sapiens
IIDEWRKKTDDLAAELDGAQRDLRNTSTDLFKAKNAQEELAEVVEGLRRENKSLSQEIKDLTDQLGEGGRSVHEMQKIIRRLEIEKEELQHALDEAEAALEAEESKVLRAQVEVSQIRSEIEKRIQEKEEEFENTRKNHARALESMQASLE

SEQ ID NO: 2 - protein, 16 aa, Homo sapiens
LQHALDEAEAALEAEE

SEQ ID NO: 3 - protein, 16 aa, Homo sapiens
LQHALDEAEAALEAEE

SEQ ID NO: 4 - protein, 20 aa, Homo sapiens
EELQHALDEAEAALEAEESK